European Patent Application EP 4 467 649 A1, published November 27, 2024. Title: Recombinantly Expressed Glutamate Oxidase. Applicant: Kikkoman Corporation. Application JP. The sequence listing filed with the application follows.

SEQUENCE LISTING (117 sequences)

SEQ ID NO: 1 - protein, 687 aa, Streptomyces sp. X-119-6
MNEMTYEQLARELLLVGPAPTNEDLKLRYLDVLIDNGLNPPGPPKRILIVGAGIAGLVAGDLLTRAGHDVTILEANANRVGGRIKTFHAKKGEPSPFADPAQYAEAGAMRLPSFHPLTLALIDKLGLKRRLFFNVDIDPQTGNQDAPVPPVFYKSFKDGKTWTNGAPSPEFKEPDKRNHTWIRTNREQVRRAQYATDPSSINEGFHLTGCETRLTVSDMVNQALEPVRDYYSVKQDDGTRVNKPFKEWLAGWADVVRDFDGYSMGRFLREYAEFSDEAVEAIGTIENMTSRLHLAFFHSFLGRSDIDPRATYWEIEGGSRMLPETLAKDLRDQIVMGQRMVRLEYYDPGRDGHHGELTGPGGPAVAIQTVPEGEPYAATQTWTGDLAIVTIPFSSLRFVKVTPPFSYKKRRAVIETHYDQATKVLLEFSRRWWEFTEADWKRELDAIAPGLYDYYQQWGEDDAEAALALPQSVRNLPTGLLGAHPSVDESRIGEEQVEYYRNSELRGGVRPATNAYGGGSTTDNPNRFMYYPSHPVPGTQGGVVLAAYSWSDDAARWDSFDDAERYGYALENLQSVHGRRIEVFYTGAGQTQSWLRDPYACGEAAVYTPHQMTAFHLDVVRPEGPVYFAGEHVSLKHAWIEGAVETAVRAAIAVNEAPVGDTGVTAAAGRRGAAAATEPMREEALTS

SEQ ID NO: 2 - DNA, 2064 bp, Streptomyces sp. X-119-6
  source 1..2064: mol_type = other DNA
atgaatgaaatgacctacgagcaattggcccgcgaattgttattggttggtccggccccgacgaacgaggatcttaaattacgctatttggatgtgctgattgataacgggctgaacccgccgggtccgcctaagcgtatcttgatcgtcggggctggtattgcaggccttgttgccggagatttgttgacccgcgctgggcatgatgttactattcttgaagctaatgccaaccgtgtgggagggcgtatcaagacgttccatgcaaaaaaaggagagccatctccattcgctgatccagcgcagtacgcggaagctggggcgatgcgtcttccttcctttcacccacttaccttggcacttatcgacaagctgggcttaaaacgccgcctgttttttaatgtagatattgacccacaaactggaaatcaagatgctccagtcccaccggtcttctataagtcttttaaggacggcaagacgtggacaaatggagccccgagccctgagtttaaagagcccgataaacgtaatcacacctggatccgtacgaatcgcgaacaagtacgccgcgcccaatacgccacagacccgagctccatcaatgaaggcttccatctgacgggatgtgagacccgccttactgtctccgacatggttaaccaagcgcttgaaccggtacgcgactattattcagtcaagcaggacgatggaactcgtgtgaataagcctttcaaagaatggcttgcagggtgggccgacgtcgtgcgtgatttcgacggttattctatgggccgcttcttacgtgaatatgccgagttttcggatgaggcagtggaagcaattggcacaattgaaaacatgacctcgcgcctgcaccttgccttttttcattcgtttttgggccgttccgatatcgatccgcgcgccacttactgggagatcgagggggggtcacgcatgcttcctgaaacactggcaaaggacctgcgcgatcagatcgttatgggtcagcgcatggtacgcttagagtactatgacccgggccgcgatggccatcatggtgagcttactgggcctgggggtccggccgtggccattcagacggttccagagggagagccttacgccgcaactcaaacgtggacaggagacctggcgattgttactatcccctttagctctttacgctttgttaaagtaacgccacccttctcttataaaaagcgccgcgcggtaattgagacccattatgatcaggccaccaaagtcttacttgaatttagccgtcgttggtgggaattcacagaggcggactggaagcgtgagcttgatgctatcgccccgggtctgtacgactattatcaacagtggggtgaagacgacgccgaagcagcgcttgcactgccgcagtcagtccgcaacttgcctaccggcttgcttggggcccacccaagcgtcgacgaatcgcgtatcggagaggagcaagttgagtattatcgtaacagcgaactgcgtggcggagtgcgccctgcgaccaatgcgtacggagggggtagtacgaccgataatcctaatcgtttcatgtactatccctcccaccccgttccaggcacgcaggggggggtcgtacttgcagcatacagttggagcgatgatgcagctcgttgggattcttttgacgatgctgagcgctatggctatgcgcttgaaaacttacagtctgtccacggccgtcgtattgaggtgttctatacaggagcgggacagacccaatcatggctgcgcgatccgtacgcatgcggcgaggcagctgtctatacaccccatcaaatgaccgcgtttcacttagatgtggtgcgtcccgaggggcccgtctattttgcgggtgagcacgtttcattaaaacatgcctggatcgagggggcggtggaaacagccgttcgtgcggcgatcgctgtaaatgaagcccccgtaggtgacactggggtcacagccgctgctgggcgccgtggggcggccgccgctactgagcctatgcgcgaggaggcgttaacttcttaa

SEQ ID NO: 3 - DNA, 708 bp, synthetic construct
  misc_feature 1..708: note = StGLOD-f1
  source 1..708: mol_type = other DNA
atgaatgaaatgacctacgagcaattggcccgcgaattgttattggttggtccggccccgacgaacgaggatcttaaattacgctatttggatgtgctgattgataacgggctgaacccgccgggtccgcctaagcgtatcttgatcgtcggggctggtattgcaggccttgttgccggagatttgttgacccgcgctgggcatgatgttactattcttgaagctaatgccaaccgtgtgggagggcgtatcaagacgttccatgcaaaaaaaggagagccatctccattcgctgatccagcgcagtacgcggaagctggggcgatgcgtcttccttcctttcacccacttaccttggcacttatcgacaagctgggcttaaaacgccgcctgttttttaatgtagatattgacccacaaactggaaatcaagatgctccagtcccaccggtcttctataagtcttttaaggacggcaagacgtggacaaatggagccccgagccctgagtttaaagagcccgataaacgtaatcacacctggatccgtacgaatcgcgaacaagtacgccgcgcccaatacgccacagacccgagctccatcaatgaaggcttccatctgacgggatgtgagacccgccttactgtctccgacatggttaaccaagcgcttgaaccggtacgcgactattattcagtcaagcaggac

SEQ ID NO: 4 - DNA, 690 bp, synthetic construct
  misc_feature 1..690: note = StGLOD-f2
  source 1..690: mol_type = other DNA
tcagtcaagcaggacgatggaactcgtgtgaataagcctttcaaagaatggcttgcagggtgggccgacgtcgtgcgtgatttcgacggttattctatgggccgcttcttacgtgaatatgccgagttttcggatgaggcagtggaagcaattggcacaattgaaaacatgacctcgcgcctgcaccttgccttttttcattcgtttttgggccgttccgatatcgatccgcgcgccacttactgggagatcgagggggggtcacgcatgcttcctgaaacactggcaaaggacctgcgcgatcagatcgttatgggtcagcgcatggtacgcttagagtactatgacccgggccgcgatggccatcatggtgagcttactgggcctgggggtccggccgtggccattcagacggttccagagggagagccttacgccgcaactcaaacgtggacaggagacctggcgattgttactatcccctttagctctttacgctttgttaaagtaacgccacccttctcttataaaaagcgccgcgcggtaattgagacccattatgatcaggccaccaaagtcttacttgaatttagccgtcgttggtgggaattcacagaggcggactggaagcgtgagcttgatgctatcgccccgggtctgtacgactattatcaacagtggggtgaagac

SEQ ID NO: 5 - DNA, 696 bp, synthetic construct
  misc_feature 1..696: note = StGLOD-f3
  source 1..696: mol_type = other DNA
cagtggggtgaagacgacgccgaagcagcgcttgcactgccgcagtcagtccgcaacttgcctaccggcttgcttggggcccacccaagcgtcgacgaatcgcgtatcggagaggagcaagttgagtattatcgtaacagcgaactgcgtggcggagtgcgccctgcgaccaatgcgtacggagggggtagtacgaccgataatcctaatcgtttcatgtactatccctcccaccccgttccaggcacgcaggggggggtcgtacttgcagcatacagttggagcgatgatgcagctcgttgggattcttttgacgatgctgagcgctatggctatgcgcttgaaaacttacagtctgtccacggccgtcgtattgaggtgttctatacaggagcgggacagacccaatcatggctgcgcgatccgtacgcatgcggcgaggcagctgtctatacaccccatcaaatgaccgcgtttcacttagatgtggtgcgtcccgaggggcccgtctattttgcgggtgagcacgtttcattaaaacatgcctggatcgagggggcggtggaaacagccgttcgtgcggcgatcgctgtaaatgaagcccccgtaggtgacactggggtcacagccgctgctgggcgccgtggggcggccgccgctactgagcctatgcgcgaggaggcgttaacttcttaa

SEQ ID NO: 6 - DNA, 40 bp, synthetic construct
  misc_feature 1..40: note = primer
  source 1..40: mol_type = other DNA
ggtcatttcattcatgaattctgtttcctgtgtgaaattg

SEQ ID NO: 7 - DNA, 38 bp, synthetic construct
  misc_feature 1..38: note = primer
  source 1..38: mol_type = other DNA
gcgttaacttcttaagcttggctgttttggcggatgag

SEQ ID NO: 8 - DNA, 30 bp, synthetic construct
  misc_feature 1..30: note = primer
  source 1..30: mol_type = other DNA
gataagaccgaagcgaccaatgcgtacgga

SEQ ID NO: 9 - DNA, 30 bp, synthetic construct
  misc_feature 1..30: note = primer
  source 1..30: mol_type = other DNA
cagcttacgataatagtcgtacagacccgg

SEQ ID NO: 10 - DNA, 30 bp, synthetic construct
  misc_feature 1..30: note = primer
  source 1..30: mol_type = other DNA
gcagagccacctgcgaccaatgcgtacgga

SEQ ID NO: 11 - DNA, 30 bp, synthetic construct
  misc_feature 1..30: note = primer
  source 1..30: mol_type = other DNA
cgcatcttgataatagtcgtacagacccgg

SEQ ID NO: 12 - protein, 638 aa, Streptomyces sp. X-119-6
MNEMTYEQLARELLLVGPAPTNEDLKLRYLDVLIDNGLNPPGPPKRILIVGAGIAGLVAGDLLTRAGHDVTILEANANRVGGRIKTFHAKKGEPSPFADPAQYAEAGAMRLPSFHPLTLALIDKLGLKRRLFFNVDIDPQTGNQDAPVPPVFYKSFKDGKTWTNGAPSPEFKEPDKRNHTWIRTNREQVRRAQYATDPSSINEGFHLTGCETRLTVSDMVNQALEPVRDYYSVKQDDGTRVNKPFKEWLAGWADVVRDFDGYSMGRFLREYAEFSDEAVEAIGTIENMTSRLHLAFFHSFLGRSDIDPRATYWEIEGGSRMLPETLAKDLRDQIVMGQRMVRLEYYDPGRDGHHGELTGPGGPAVAIQTVPEGEPYAATQTWTGDLAIVTIPFSSLRFVKVTPPFSYKKRRAVIETHYDQATKVLLEFSRRWWEFTEADWKRELDAIAPGLYDYYRKLDKTEATNAYGGGSTTDNPNRFMYYPSHPVPGTQGGVVLAAYSWSDDAARWDSFDDAERYGYALENLQSVHGRRIEVFYTGAGQTQSWLRDPYACGEAAVYTPHQMTAFHLDVVRPEGPVYFAGEHVSLKHAWIEGAVETAVRAAIAVNEAPVGDTGVTAAAGRRGAAAATEPMREEALTS

SEQ ID NO: 13 - protein, 638 aa, Streptomyces sp. X-119-6
MNEMTYEQLARELLLVGPAPTNEDLKLRYLDVLIDNGLNPPGPPKRILIVGAGIAGLVAGDLLTRAGHDVTILEANANRVGGRIKTFHAKKGEPSPFADPAQYAEAGAMRLPSFHPLTLALIDKLGLKRRLFFNVDIDPQTGNQDAPVPPVFYKSFKDGKTWTNGAPSPEFKEPDKRNHTWIRTNREQVRRAQYATDPSSINEGFHLTGCETRLTVSDMVNQALEPVRDYYSVKQDDGTRVNKPFKEWLAGWADVVRDFDGYSMGRFLREYAEFSDEAVEAIGTIENMTSRLHLAFFHSFLGRSDIDPRATYWEIEGGSRMLPETLAKDLRDQIVMGQRMVRLEYYDPGRDGHHGELTGPGGPAVAIQTVPEGEPYAATQTWTGDLAIVTIPFSSLRFVKVTPPFSYKKRRAVIETHYDQATKVLLEFSRRWWEFTEADWKRELDAIAPGLYDYYQDAAEPPATNAYGGGSTTDNPNRFMYYPSHPVPGTQGGVVLAAYSWSDDAARWDSFDDAERYGYALENLQSVHGRRIEVFYTGAGQTQSWLRDPYACGEAAVYTPHQMTAFHLDVVRPEGPVYFAGEHVSLKHAWIEGAVETAVRAAIAVNEAPVGDTGVTAAAGRRGAAAATEPMREEALTS

SEQ ID NO: 14 - DNA, 30 bp, synthetic construct
  misc_feature 1..30: note = primer
  source 1..30: mol_type = other DNA
cgtcttgatacgccctcccacacggttggc

SEQ ID NO: 15 - DNA, 30 bp, synthetic construct
  misc_feature 1..30: note = primer
  source 1..30: mol_type = other DNA
cgtatcaagacgtaccatgcaaaaaaagga

SEQ ID NO: 16 - DNA, 30 bp, synthetic construct
  misc_feature 1..30: note = primer
  source 1..30: mol_type = other DNA
ctgcgctggatcagcgaatggagatggctc

SEQ ID NO: 17 - DNA, 30 bp, synthetic construct
  misc_feature 1..30: note = primer
  source 1..30: mol_type = other DNA
gatccagcgcagttcgcggaagctggggcg

SEQ ID NO: 18 - DNA, 30 bp, synthetic construct
  misc_feature 1..30: note = primer
  source 1..30: mol_type = other DNA
gatccagcgcagttagcggaagctggggcg

SEQ ID NO: 19 - DNA, 30 bp, synthetic construct
  misc_feature 1..30: note = primer
  source 1..30: mol_type = other DNA
gatccagcgcaggtcgcggaagctggggcg

SEQ ID NO: 20 - DNA, 30 bp, synthetic construct
  misc_feature 1..30: note = primer
  source 1..30: mol_type = other DNA
gatccagcgcagatcgcggaagctggggcg

SEQ ID NO: 21 - DNA, 30 bp, synthetic construct
  misc_feature 1..30: note = primer
  source 1..30: mol_type = other DNA
gatccagcgcagatggcggaagctggggcg

SEQ ID NO: 22 - DNA, 30 bp, synthetic construct
  misc_feature 1..30: note = primer
  source 1..30: mol_type = other DNA
aaacaggcggcgttttaagcccagcttgtc

SEQ ID NO: 23 - DNA, 30 bp, synthetic construct
  misc_feature 1..30: note = primer
  source 1..30: mol_type = other DNA
cgccgcctgttttataatgtagatattgac

SEQ ID NO: 24 - DNA, 30 bp, synthetic construct
  misc_feature 1..30: note = primer
  source 1..30: mol_type = other DNA
cgccgcctgtttttaaatgtagatattgac

SEQ ID NO: 25 - DNA, 30 bp, synthetic construct
  misc_feature 1..30: note = primer
  source 1..30: mol_type = other DNA
aaaggcaaggtgcaggcgcgaggtcatgtt

SEQ ID NO: 26 - DNA, 30 bp, synthetic construct
  misc_feature 1..30: note = primer
  source 1..30: mol_type = other DNA
caccttgcctttttacattcgtttttgggc

SEQ ID NO: 27 - DNA, 30 bp, synthetic construct
  misc_feature 1..30: note = primer
  source 1..30: mol_type = other DNA
caccttgcctttgttcattcgtttttgggc

SEQ ID NO: 28 - DNA, 30 bp, synthetic construct
  misc_feature 1..30: note = primer
  source 1..30: mol_type = other DNA
caccttgcctttattcattcgtttttgggc

SEQ ID NO: 29 - DNA, 30 bp, synthetic construct
  misc_feature 1..30: note = primer
  source 1..30: mol_type = other DNA
caccttgcctttatgcattcgtttttgggc

SEQ ID NO: 30 - DNA, 30 bp, synthetic construct
  misc_feature 1..30: note = primer
  source 1..30: mol_type = other DNA
aggctctccctctggaaccgtctgaatggc

SEQ ID NO: 31 - DNA, 30 bp, synthetic construct
  misc_feature 1..30: note = primer
  source 1..30: mol_type = other DNA
gagggagagcctttcgccgcaactcaaacg

SEQ ID NO: 32 - DNA, 30 bp, synthetic construct
  misc_feature 1..30: note = primer
  source 1..30: mol_type = other DNA
gagggagagcctttagccgcaactcaaacg

SEQ ID NO: 33 - DNA, 30 bp, synthetic construct
  misc_feature 1..30: note = primer
  source 1..30: mol_type = other DNA
gagggagagcctatcgccgcaactcaaacg

SEQ ID NO: 34 - DNA, 30 bp, synthetic construct
  misc_feature 1..30: note = primer
  source 1..30: mol_type = other DNA
gagggagagcctatggccgcaactcaaacg

SEQ ID NO: 35 - DNA, 30 bp, synthetic construct
  misc_feature 1..30: note = primer
  source 1..30: mol_type = other DNA
ggggatagtaacaatcgccaggtctcctgt

SEQ ID NO: 36 - DNA, 30 bp, synthetic construct
  misc_feature 1..30: note = primer
  source 1..30: mol_type = other DNA
gttactatccccttaagctctttacgcttt

SEQ ID NO: 37 - DNA, 30 bp, synthetic construct
  misc_feature 1..30: note = primer
  source 1..30: mol_type = other DNA
gttactatccccgttagctctttacgcttt

SEQ ID NO: 38 - DNA, 30 bp, synthetic construct
  misc_feature 1..30: note = primer
  source 1..30: mol_type = other DNA
gttactatccccattagctctttacgcttt

SEQ ID NO: 39 - DNA, 30 bp, synthetic construct
  misc_feature 1..30: note = primer
  source 1..30: mol_type = other DNA
gttactatccccatgagctctttacgcttt

SEQ ID NO: 40 - DNA, 30 bp, synthetic construct
  misc_feature 1..30: note = primer
  source 1..30: mol_type = other DNA
ttcaagtaagactttggtggcctgatcata

SEQ ID NO: 41 - DNA, 30 bp, synthetic construct
  misc_feature 1..30: note = primer
  source 1..30: mol_type = other DNA
gtcttacttgaatatagccgtcgttggtgg

SEQ ID NO: 42 - DNA, 30 bp, synthetic construct
  misc_feature 1..30: note = primer
  source 1..30: mol_type = other DNA
gtcttacttgaaatgagccgtcgttggtgg

SEQ ID NO: 43 - DNA, 30 bp, synthetic construct
  misc_feature 1..30: note = primer
  source 1..30: mol_type = other DNA
cgcattggtcgcaggtggctctgccgcatc

SEQ ID NO: 44 - DNA, 30 bp, synthetic construct
  misc_feature 1..30: note = primer
  source 1..30: mol_type = other DNA
gcgaccaatgcgttcggagggggtagtacg

SEQ ID NO: 45 - DNA, 30 bp, synthetic construct
  misc_feature 1..30: note = primer
  source 1..30: mol_type = other DNA
gcgctcagcatcgtcaaaagaatcccaacg

SEQ ID NO: 46 - DNA, 30 bp, synthetic construct
  misc_feature 1..30: note = primer
  source 1..30: mol_type = other DNA
gatgctgagcgctttggctatgcgcttgaa

SEQ ID NO: 47 - DNA, 30 bp, synthetic construct
  misc_feature 1..30: note = primer
  source 1..30: mol_type = other DNA
gatgctgagcgcttaggctatgcgcttgaa

SEQ ID NO: 48 - DNA, 30 bp, synthetic construct
  misc_feature 1..30: note = primer
  source 1..30: mol_type = other DNA
gatgctgagcgcgttggctatgcgcttgaa

SEQ ID NO: 49 - DNA, 30 bp, synthetic construct
  misc_feature 1..30: note = primer
  source 1..30: mol_type = other DNA
gatgctgagcgcatgggctatgcgcttgaa

SEQ ID NO: 50 - DNA, 30 bp, synthetic construct
  misc_feature 1..30: note = primer
  source 1..30: mol_type = other DNA
gccatagcgctcagcatcgtcaaaagaatc

SEQ ID NO: 51 - DNA, 30 bp, synthetic construct
  misc_feature 1..30: note = primer
  source 1..30: mol_type = other DNA
gagcgctatggcattgcgcttgaaaactta

SEQ ID NO: 52 - DNA, 30 bp, synthetic construct
  misc_feature 1..30: note = primer
  source 1..30: mol_type = other DNA
gagcgctatggcatggcgcttgaaaactta

SEQ ID NO: 53 - DNA, 30 bp, synthetic construct
  misc_feature 1..30: note = primer
  source 1..30: mol_type = other DNA
gaacacctcaatacgacggccgtggacaga

SEQ ID NO: 54 - DNA, 30 bp, synthetic construct
  misc_feature 1..30: note = primer
  source 1..30: mol_type = other DNA
attgaggtgttcttaacaggagcgggacag

SEQ ID NO: 55 - DNA, 30 bp, synthetic construct
  misc_feature 1..30: note = primer
  source 1..30: mol_type = other DNA
attgaggtgttcatgacaggagcgggacag

SEQ ID NO: 56 - DNA, 30 bp, synthetic construct
  misc_feature 1..30: note = primer
  source 1..30: mol_type = other DNA
cgcggtcatttgatggggtgtatagacagc

SEQ ID NO: 57 - DNA, 30 bp, synthetic construct
  misc_feature 1..30: note = primer
  source 1..30: mol_type = other DNA
caaatgaccgcgttacacttagatgtggtg

SEQ ID NO: 58 - protein, 690 aa, Streptomyces sp. MOE7
MDDKTYQQLARELLLVGPEPANEDLKLRYLDVLIDNGLEPPVDRKRILIVGAGIAGLVAGHLLTRAGHDVTILEANANRVGGRIKTFHAKKGEPAPFTDPAQYAEAGAMRLPSFHPLTLALIDKLGLKRRLFFNVDIDPKTGNQGAALPPVVYKSFKDGKTWTYGKPSPEFREPDKRNHTWIRTNRTQVRRAQYVKDPSAINEGFHLTGCESRLTVSDMVNQALEPVRDYYSVLQSDGRRVNKPFKEWLDGWAGVIRDFDGFSMGRFLREYAGFSDEAVEAIGTIENMTSRLHLAFFHSFLGRSDIDPSATYWEIEGGSRQLPEALAKDLRDQIVMGQRMVRLEYYDPGRDGHHGGLAGPSGPAVAIETVPENEPSAEPQTWTADLAIVTVPFSSLRFVAVTPPFSYKKRRAVIETHYDQATKVLLEFSRRWWEFTEEDWKRELDAIAPGLYEYYQRWGEDDAEAALTVPESVRNLPTGLLGAHPSVDEQLIDDEQVEYLRNSTLRGGVRPATQVHGGGSTTDNPNRFMYYPSHAVPGSKGGVVLAAYSWSDDAARWDSFDDAERYGYALENLQSVHGRRIEVFYTGAGQTQSWLRDPYACGEAAVYTPHQMTSFHLDVVRPEGPVYFAGEHVSLKHAWIEGAVETAVRAAIAVNEAPVPYDTAAARAEAPRERAGTASATRTREKAVTS

SEQ ID NO: 59 - protein, 641 aa, Streptomyces sp. MOE7
MDDKTYQQLARELLLVGPEPANEDLKLRYLDVLIDNGLEPPVDRKRILIVGAGIAGLVAGHLLTRAGHDVTILEANANRVGGRIKTFHAKKGEPAPFTDPAQYAEAGAMRLPSFHPLTLALIDKLGLKRRLFFNVDIDPKTGNQGAALPPVVYKSFKDGKTWTYGKPSPEFREPDKRNHTWIRTNRTQVRRAQYVKDPSAINEGFHLTGCESRLTVSDMVNQALEPVRDYYSVLQSDGRRVNKPFKEWLDGWAGVIRDFDGFSMGRFLREYAGFSDEAVEAIGTIENMTSRLHLAFFHSFLGRSDIDPSATYWEIEGGSRQLPEALAKDLRDQIVMGQRMVRLEYYDPGRDGHHGGLAGPSGPAVAIETVPENEPSAEPQTWTADLAIVTVPFSSLRFVAVTPPFSYKKRRAVIETHYDQATKVLLEFSRRWWEFTEEDWKRELDAIAPGLYEYYQDAAEPPATQVHGGGSTTDNPNRFMYYPSHAVPGSKGGVVLAAYSWSDDAARWDSFDDAERYGYALENLQSVHGRRIEVFYTGAGQTQSWLRDPYACGEAAVYTPHQMTSFHLDVVRPEGPVYFAGEHVSLKHAWIEGAVETAVRAAIAVNEAPVPYDTAAARAEAPRERAGTASATRTREKAVTS

SEQ ID NO: 60 - protein, 641 aa, Streptomyces sp. MOE7
MDDKTYQQLARELLLVGPEPANEDLKLRYLDVLIDNGLEPPVDRKRILIVGAGIAGLVAGHLLTRAGHDVTILEANANRVGGRIKTYHAKKGEPAPFTDPAQIAEAGAMRLPSFHPLTLALIDKLGLKRRLFYNVDIDPKTGNQGAALPPVVYKSFKDGKTWTYGKPSPEFREPDKRNHTWIRTNRTQVRRAQYVKDPSAINEGFHLTGCESRLTVSDMVNQALEPVRDYYSVLQSDGRRVNKPFKEWLDGWAGVIRDFDGFSMGRFLREYAGFSDEAVEAIGTIENMTSRLHLAFMHSFLGRSDIDPSATYWEIEGGSRQLPEALAKDLRDQIVMGQRMVRLEYYDPGRDGHHGGLAGPSGPAVAIETVPENEPSAEPQTWTADLAIVTVPLSSLRFVAVTPPFSYKKRRAVIETHYDQATKVLLEYSRRWWEFTEEDWKRELDAIAPGLYEYYQDAAEPPATQVHGGGSTTDNPNRFMYYPSHAVPGSKGGVVLAAYSWSDDAARWDSFDDAERFGYALENLQSVHGRRIEVFLTGAGQTQSWLRDPYACGEAAVYTPHQMTSFHLDVVRPEGPVYFAGEHVSLKHAWIEGAVETAVRAAIAVNEAPVPYDTAAARAEAPRERAGTASATRTREKAVTS

SEQ ID NO: 61 - DNA, 1926 bp, Streptomyces sp. MOE7
  source 1..1926: mol_type = other DNA
atggacgacaagacctatcagcagttagcacgcgaactgctgcttgtagggcccgagccagcgaatgaagatcttaaattgcgctatttagacgtacttattgataacgggctggagcccccagtcgatcgtaaacgtatcttaattgtgggggcagggatcgccggcctggtcgcgggacatttgttgacacgcgcgggacacgatgtcaccatcctggaggcgaatgcaaatcgcgttggaggtcgcattaagacatatcatgcaaagaaaggcgaaccggcccccttcaccgacccggctcaaattgcagaggcgggagctatgcgtttgccttcattccatcccttaacgttagcgctgattgataaattagggttgaagcgtcgcttgttctataatgttgacattgaccctaagacgggcaatcaaggtgcagcattgccgcctgtcgtttacaagagctttaaggacggtaaaacttggacgtatggtaaaccttctccggaattccgtgaaccagacaaacgtaaccacacttggattcgtaccaatcgcactcaagtacgtcgcgcccagtatgtgaaggacccgagtgcgattaacgaagggttccatttaaccgggtgcgagtcgcgtttgacagtttctgatatggtgaaccaagctttagaaccggttcgtgactactattctgtattgcagagcgacgggcgccgcgtaaataagccatttaaggagtggttagacggctgggccggtgtaatccgcgatttcgacggattctcaatgggacgttttctgcgcgagtacgctgggttttcggacgaggcggtagaagcaatcggtaccatcgagaatatgacaagtcgtttgcatttggcatttatgcacagcttcttaggtcgcagtgacattgaccccagcgcgacatattgggagattgaaggcggtagccgtcagctgcctgaggctctggcaaaagacctgcgtgatcagattgtaatgggccaacgcatggtgcgtttagagtactacgacccaggacgtgatggacaccatggaggtctggcaggaccctctggtcctgcggttgcaatcgaaactgtacccgagaacgagccaagtgcagagccgcagacgtggactgcggacctggcgattgtcactgtaccactttcgtctcttcgctttgttgcggtgactcccccattcagttataaaaaacgtcgtgcagttatcgaaactcactatgatcaggcaacaaaagtgctgttagagtattctcgtcgctggtgggagtttacagaagaggactggaagcgtgagttggacgcgattgcccccggcctgtatgaatactaccaggatgctgcagaaccgccggcaactcaagttcatggaggaggttcaacaactgacaatccaaaccgttttatgtattatccgagtcacgcggtgcctggttctaagggtggtgtggttttggccgcgtatagttggagtgacgatgcagcgcgttgggattcctttgatgacgccgaacgttttggctacgccctggaaaaccttcaatcggtccatggccgccgcatcgaggtctttttaactggagctggacaaactcagtcatggttgcgcgacccctacgcctgcggtgaggccgcagtttacacaccacatcagatgacatcttttcacttagacgtagtgcgcccggaggggccagtatactttgcgggagagcatgtctctcttaagcatgcgtggatcgagggggccgttgaaaccgcggtccgtgctgcgatcgcggttaacgaagcccccgtaccatacgacacagctgctgctcgtgcggaggcccctcgcgaacgtgccggtacagcatcagccactcgcacgcgcgagaaggccgtgacttcctaa

SEQ ID NO: 62 - DNA, 655 bp, synthetic construct
  misc_feature 1..655: note = M7GLOD delta 49C-T8-f1
  source 1..655: mol_type = other DNA
ggagatatacatatggacgacaagacctatcagcagttagcacgcgaactgctgcttgtagggcccgagccagcgaatgaagatcttaaattgcgctatttagacgtacttattgataacgggctggagcccccagtcgatcgtaaacgtatcttaattgtgggggcagggatcgccggcctggtcgcgggacatttgttgacacgcgcgggacacgatgtcaccatcctggaggcgaatgcaaatcgcgttggaggtcgcattaagacatatcatgcaaagaaaggcgaaccggcccccttcaccgacccggctcaaattgcagaggcgggagctatgcgtttgccttcattccatcccttaacgttagcgctgattgataaattagggttgaagcgtcgcttgttctataatgttgacattgaccctaagacgggcaatcaaggtgcagcattgccgcctgtcgtttacaagagctttaaggacggtaaaacttggacgtatggtaaaccttctccggaattccgtgaaccagacaaacgtaaccacacttggattcgtaccaatcgcactcaagtacgtcgcgcccagtatgtgaaggacccgagtgcgattaacgaagggttccatttaaccgggtgcgagtcgcgtttga

SEQ ID NO: 63 - DNA, 670 bp, synthetic construct
  misc_feature 1..670: note = M7GLOD delta 49C-T8-f2
  source 1..670: mol_type = other DNA
gcgagtcgcgtttgacagtttctgatatggtgaaccaagctttagaaccggttcgtgactactattctgtattgcagagcgacgggcgccgcgtaaataagccatttaaggagtggttagacggctgggccggtgtaatccgcgatttcgacggattctcaatgggacgttttctgcgcgagtacgctgggttttcggacgaggcggtagaagcaatcggtaccatcgagaatatgacaagtcgtttgcatttggcatttatgcacagcttcttaggtcgcagtgacattgaccccagcgcgacatattgggagattgaaggcggtagccgtcagctgcctgaggctctggcaaaagacctgcgtgatcagattgtaatgggccaacgcatggtgcgtttagagtactacgacccaggacgtgatggacaccatggaggtctggcaggaccctctggtcctgcggttgcaatcgaaactgtacccgagaacgagccaagtgcagagccgcagacgtggactgcggacctggcgattgtcactgtaccactttcgtctcttcgctttgttgcggtgactcccccattcagttataaaaaacgtcgtgcagttatcgaaactcactatgatcaggcaacaaaagtgctgttagagtattctcgtcgctggtg

SEQ ID NO: 64 - DNA, 655 bp, synthetic construct
  misc_feature 1..655: note = M7GLOD delta 49C-T8-f3
  source 1..655: mol_type = other DNA
ttctcgtcgctggtgggagtttacagaagaggactggaagcgtgagttggacgcgattgcccccggcctgtatgaatactaccaggatgctgcagaaccgccggcaactcaagttcatggaggaggttcaacaactgacaatccaaaccgttttatgtattatccgagtcacgcggtgcctggttctaagggtggtgtggttttggccgcgtatagttggagtgacgatgcagcgcgttgggattcctttgatgacgccgaacgttttggctacgccctggaaaaccttcaatcggtccatggccgccgcatcgaggtctttttaactggagctggacaaactcagtcatggttgcgcgacccctacgcctgcggtgaggccgcagtttacacaccacatcagatgacatcttttcacttagacgtagtgcgcccggaggggccagtatactttgcgggagagcatgtctctcttaagcatgcgtggatcgagggggccgttgaaaccgcggtccgtgctgcgatcgcggttaacgaagcccccgtaccatacgacacagctgctgctcgtgcggaggcccctcgcgaacgtgccggtacagcatcagccactcgcacgcgcgagaaggccgtgacttcctaacaaagcccgaaa

SEQ ID NO: 65 - DNA, 24 bp, synthetic construct
  misc_feature 1..24: note = primer
  source 1..24: mol_type = other DNA
catatgtatatctccttcttaaag

SEQ ID NO: 66 - DNA, 20 bp, synthetic construct
  misc_feature 1..20: note = primer
  source 1..20: mol_type = other DNA
taacaaagcccgaaaggaag

SEQ ID NO: 67 - DNA, 30 bp, synthetic construct
  misc_feature 1..30: note = primer
  source 1..30: mol_type = other DNA
atcgaggtcttttatactggagctggacaa

SEQ ID NO: 68 - DNA, 30 bp, synthetic construct
  misc_feature 1..30: note = primer
  source 1..30: mol_type = other DNA
aaagacctcgatgcggcggccatggaccga

SEQ ID NO: 69 - protein, 641 aa, Streptomyces sp. MOE7
MDDKTYQQLARELLLVGPEPANEDLKLRYLDVLIDNGLEPPVDRKRILIVGAGIAGLVAGHLLTRAGHDVTILEANANRVGGRIKTYHAKKGEPAPFTDPAQIAEAGAMRLPSFHPLTLALIDKLGLKRRLFYNVDIDPKTGNQGAALPPVVYKSFKDGKTWTYGKPSPEFREPDKRNHTWIRTNRTQVRRAQYVKDPSAINEGFHLTGCESRLTVSDMVNQALEPVRDYYSVLQSDGRRVNKPFKEWLDGWAGVIRDFDGFSMGRFLREYAGFSDEAVEAIGTIENMTSRLHLAFMHSFLGRSDIDPSATYWEIEGGSRQLPEALAKDLRDQIVMGQRMVRLEYYDPGRDGHHGGLAGPSGPAVAIETVPENEPSAEPQTWTADLAIVTVPLSSLRFVAVTPPFSYKKRRAVIETHYDQATKVLLEYSRRWWEFTEEDWKRELDAIAPGLYEYYQDAAEPPATQVHGGGSTTDNPNRFMYYPSHAVPGSKGGVVLAAYSWSDDAARWDSFDDAERFGYALENLQSVHGRRIEVFYTGAGQTQSWLRDPYACGEAAVYTPHQMTSFHLDVVRPEGPVYFAGEHVSLKHAWIEGAVETAVRAAIAVNEAPVPYDTAAARAEAPRERAGTASATRTREKAVTS

SEQ ID NO: 70 - DNA, 27 bp, synthetic construct
  misc_feature 1..27: note = primer
  source 1..27: mol_type = other DNA
attggtacgaatccaagtgtggttacg

SEQ ID NO: 71 - DNA, 30 bp, synthetic construct
  misc_feature 1..30: note = primer
  source 1..30: mol_type = other DNA
attcgtaccaatggcactcaagtacgtcgc

SEQ ID NO: 72 - DNA, 30 bp, synthetic construct
  misc_feature 1..30: note = primer
  source 1..30: mol_type = other DNA
attcgtaccaatgcgactcaagtacgtcgc

SEQ ID NO: 73 - DNA, 30 bp, synthetic construct
  misc_feature 1..30: note = primer
  source 1..30: mol_type = other DNA
attcgtaccaattgcactcaagtacgtcgc

SEQ ID NO: 74 - DNA, 30 bp, synthetic construct
  misc_feature 1..30: note = primer
  source 1..30: mol_type = other DNA
attcgtaccaatctgactcaagtacgtcgc

SEQ ID NO: 75 - DNA, 30 bp, synthetic construct
  misc_feature 1..30: note = primer
  source 1..30: mol_type = other DNA
attcgtaccaatatgactcaagtacgtcgc

SEQ ID NO: 76 - DNA, 30 bp, synthetic construct
  misc_feature 1..30: note = primer
  source 1..30: mol_type = other DNA
attcgtaccaattttactcaagtacgtcgc

SEQ ID NO: 77 - DNA, 30 bp, synthetic construct
  misc_feature 1..30: note = primer
  source 1..30: mol_type = other DNA
attcgtaccaattatactcaagtacgtcgc

SEQ ID NO: 78 - DNA, 30 bp, synthetic construct
  misc_feature 1..30: note = primer
  source 1..30: mol_type = other DNA
attcgtaccaatagcactcaagtacgtcgc

SEQ ID NO: 79 - DNA, 30 bp, synthetic construct
  misc_feature 1..30: note = primer
  source 1..30: mol_type = other DNA
attcgtaccaataccactcaagtacgtcgc

SEQ ID NO: 80 - DNA, 30 bp, synthetic construct
  misc_feature 1..30: note = primer
  source 1..30: mol_type = other DNA
attcgtaccaataacactcaagtacgtcgc

SEQ ID NO: 81 - DNA, 30 bp, synthetic construct
  misc_feature 1..30: note = primer
  source 1..30: mol_type = other DNA
attcgtaccaatcagactcaagtacgtcgc

SEQ ID NO: 82 - DNA, 30 bp, synthetic construct
  misc_feature 1..30: note = primer
  source 1..30: mol_type = other DNA
attcgtaccaatcatactcaagtacgtcgc

SEQ ID NO: 83 - DNA, 30 bp, synthetic construct
  misc_feature 1..30: note = primer
  source 1..30: mol_type = other DNA
attcgtaccaatgatactcaagtacgtcgc

SEQ ID NO: 84 - DNA, 30 bp, synthetic construct
  misc_feature 1..30: note = primer
  source 1..30: mol_type = other DNA
attcgtaccaatgaaactcaagtacgtcgc

SEQ ID NO: 85 - DNA, 2073 bp, synthetic construct
  misc_feature 1..2073: note = M7GLOD
  source 1..2073: mol_type = other DNA
atggacgacaagacctatcagcagttagcacgcgaactgctgcttgtagggcccgagccagcgaatgaagatcttaaattgcgctatttagacgtacttattgataacgggctggagcccccagtcgatcgtaaacgtatcttaattgtgggggcagggatcgccggcctggtcgcgggacatttgttgacacgcgcgggacacgatgtcaccatcctggaggcgaatgcaaatcgcgttggaggtcgcattaagacatttcatgcaaagaaaggcgaaccggcccccttcaccgacccggctcaatatgcagaggcgggagctatgcgtttgccttcattccatcccttaacgttagcgctgattgataaattagggttgaagcgtcgcttgttctttaatgttgacattgaccctaagacgggcaatcaaggtgcagcattgccgcctgtcgtttacaagagctttaaggacggtaaaacttggacgtatggtaaaccttctccggaattccgtgaaccagacaaacgtaaccacacttggattcgtaccaatcgcactcaagtacgtcgcgcccagtatgtgaaggacccgagtgcgattaacgaagggttccatttaaccgggtgcgagtcgcgtttgacagtttctgatatggtgaaccaagctttagaaccggttcgtgactactattctgtattgcagagcgacgggcgccgcgtaaataagccatttaaggagtggttagacggctgggccggtgtaatccgcgatttcgacggattctcaatgggacgttttctgcgcgagtacgctgggttttcggacgaggcggtagaagcaatcggtaccatcgagaatatgacaagtcgtttgcatttggcattttttcacagcttcttaggtcgcagtgacattgaccccagcgcgacatattgggagattgaaggcggtagccgtcagctgcctgaggctctggcaaaagacctgcgtgatcagattgtaatgggccaacgcatggtgcgtttagagtactacgacccaggacgtgatggacaccatggaggtctggcaggaccctctggtcctgcggttgcaatcgaaactgtacccgagaacgagccaagtgcagagccgcagacgtggactgcggacctggcgattgtcactgtaccattttcgtctcttcgctttgttgcggtgactcccccattcagttataaaaaacgtcgtgcagttatcgaaactcactatgatcaggcaacaaaagtgctgttagagttttctcgtcgctggtgggagtttacagaagaggactggaagcgtgagttggacgcgattgcccccggcctgtatgaatactaccagcgttggggcgaggacgatgccgaagcagcccttacggtacccgaaagtgtacgcaatcttccaacgggattgttaggggcccatccttccgttgacgagcaactgattgatgacgagcaggtagagtatctgcgtaattcaacattgcgtggaggcgtacgcccggcaactcaagttcatggaggaggttcaacaactgacaatccaaaccgttttatgtattatccgagtcacgcggtgcctggttctaagggtggtgtggttttggccgcgtatagttggagtgacgatgcagcgcgttgggattcctttgatgacgccgaacgttatggctacgccctggaaaaccttcaatcggtccatggccgccgcatcgaggtcttttatactggagctggacaaactcagtcatggttgcgcgacccctacgcctgcggtgaggccgcagtttacacaccacatcagatgacatcttttcacttagacgtagtgcgcccggaggggccagtatactttgcgggagagcatgtctctcttaagcatgcgtggatcgagggggccgttgaaaccgcggtccgtgctgcgatcgcggttaacgaagcccccgtaccatacgacacagctgctgctcgtgcggaggcccctcgcgaacgtgccggtacagcatcagccactcgcacgcgcgagaaggccgtgacttcctaa

SEQ ID NO: 86 - DNA, 2097 bp, synthetic construct
  misc_feature 1..2097: note = Artificial DNA fragment
  source 1..2097: mol_type = other DNA
ggagatatacatatggacgacaagacctatcagcagttagcacgcgaactgctgcttgtagggcccgagccagcgaatgaagatcttaaattgcgctatttagacgtacttattgataacgggctggagcccccagtcgatcgtaaacgtatcttaattgtgggggcagggatcgccggcctggtcgcgggacatttgttgacacgcgcgggacacgatgtcaccatcctggaggcgaatgcaaatcgcgttggaggtcgcattaagacatttcatgcaaagaaaggcgaaccggcccccttcaccgacccggctcaatatgcagaggcgggagctatgcgtttgccttcattccatcccttaacgttagcgctgattgataaattagggttgaagcgtcgcttgttctttaatgttgacattgaccctaagacgggcaatcaaggtgcagcattgccgcctgtcgtttacaagagctttaaggacggtaaaacttggacgtatggtaaaccttctccggaattccgtgaaccagacaaacgtaaccacacttggattcgtaccaatcgcactcaagtacgtcgcgcccagtatgtgaaggacccgagtgcgattaacgaagggttccatttaaccgggtgcgagtcgcgtttgacagtttctgatatggtgaaccaagctttagaaccggttcgtgactactattctgtattgcagagcgacgggcgccgcgtaaataagccatttaaggagtggttagacggctgggccggtgtaatccgcgatttcgacggattctcaatgggacgttttctgcgcgagtacgctgggttttcggacgaggcggtagaagcaatcggtaccatcgagaatatgacaagtcgtttgcatttggcattttttcacagcttcttaggtcgcagtgacattgaccccagcgcgacatattgggagattgaaggcggtagccgtcagctgcctgaggctctggcaaaagacctgcgtgatcagattgtaatgggccaacgcatggtgcgtttagagtactacgacccaggacgtgatggacaccatggaggtctggcaggaccctctggtcctgcggttgcaatcgaaactgtacccgagaacgagccaagtgcagagccgcagacgtggactgcggacctggcgattgtcactgtaccattttcgtctcttcgctttgttgcggtgactcccccattcagttataaaaaacgtcgtgcagttatcgaaactcactatgatcaggcaacaaaagtgctgttagagttttctcgtcgctggtgggagtttacagaagaggactggaagcgtgagttggacgcgattgcccccggcctgtatgaatactaccagcgttggggcgaggacgatgccgaagcagcccttacggtacccgaaagtgtacgcaatcttccaacgggattgttaggggcccatccttccgttgacgagcaactgattgatgacgagcaggtagagtatctgcgtaattcaacattgcgtggaggcgtacgcccggcaactcaagttcatggaggaggttcaacaactgacaatccaaaccgttttatgtattatccgagtcacgcggtgcctggttctaagggtggtgtggttttggccgcgtatagttggagtgacgatgcagcgcgttgggattcctttgatgacgccgaacgttatggctacgccctggaaaaccttcaatcggtccatggccgccgcatcgaggtcttttatactggagctggacaaactcagtcatggttgcgcgacccctacgcctgcggtgaggccgcagtttacacaccacatcagatgacatcttttcacttagacgtagtgcgcccggaggggccagtatactttgcgggagagcatgtctctcttaagcatgcgtggatcgagggggccgttgaaaccgcggtccgtgctgcgatcgcggttaacgaagcccccgtaccatacgacacagctgctgctcgtgcggaggcccctcgcgaacgtgccggtacagcatcagccactcgcacgcgcgagaaggccgtgacttcctaacaaagcccgaaa

SEQ ID NO: 87 - protein, 689 aa, Streptomyces sp. MOE7
MDDKTYQQLARELLLVGPEPANEDLKLRYLDVLIDNGLEPPVDRKRILIVGAGIAGLVAGHLLTRAGHDVTILEANANRVGGRIKTYHAKKGEPAPFTDPAQIAEAGAMRLPSFHPLTLALIDKLGLKRRLFNVDIDPKTGNQGAALPPVVYKSFKDGKTWTYGKPSPEFREPDKRNHTWIRTNRTQVRRAQYVKDPSAINEGFHLTGCESRLTVSDMVNQALEPVRDYYSVLQSDGRRVNKPFKEWLDGWAGVIRDFDGFSMGRFLREYAGFSDEAVEAIGTIENMTSRLHLAFMHSFLGRSDIDPSATYWEIEGGSRQLPEALAKDLRDQIVMGQRMVRLEYYDPGRDGHHGGLAGPSGPAVAIETVPENEPSAEPQTWTADLAIVTVPLSSLRFVAVTPPFSYKKRRAVIETHYDQATKVLLEYSRRWWEFTEEDWKRELDAIAPGLYEYYQRWGEDDAEAALTVPESVRNLPTGLLGAHPSVDEQLIDDEQVEYLRNSTLRGGVRPATQVHGGGSTTDNPNRFMYYPSHAVPGSKGGVVLAAYSWSDDAARWDSFDDAERFGYALENLQSVHGRRIEVFLTGAGQTQSWLRDPYACGEAAVYTPHQMTSFHLDVVRPEGPVYFAGEHVSLKHAWIEGAVETAVRAAIAVNEAPVPYDTAAARAEAPRERAGTASATRTREKAVTS

SEQ ID NO: 88 - DNA, 19 bp, synthetic construct
  misc_feature 1..19: note = primer
  source 1..19: mol_type = other DNA
ccgtcgttggtgggaattc

SEQ ID NO: 89 - DNA, 20 bp, synthetic construct
  misc_feature 1..20: note = primer
  source 1..20: mol_type = other DNA
gcgctcagcatcgtcaaaag

SEQ ID NO: 90 - DNA, 20 bp, synthetic construct
  misc_feature 1..20: note = primer
  source 1..20: mol_type = other DNA
cttttgacgatgctgagcgc

SEQ ID NO: 91 - DNA, 19 bp, synthetic construct
  misc_feature 1..19: note = primer
  source 1..19: mol_type = other DNA
gaattcccaccaacgacgg

SEQ ID NO: 92 - DNA, 30 bp, synthetic construct
  misc_feature 1..30: note = primer
  source 1..30: mol_type = other DNA
gtacgcccggcaactcaagttcatggagga

SEQ ID NO: 93 - DNA, 30 bp, synthetic construct
  misc_feature 1..30: note = primer
  source 1..30: mol_type = other DNA
aagattgcgtacactttcgggtaccgtaag

SEQ ID NO: 94 - DNA, 30 bp, synthetic construct
  misc_feature 1..30: note = primer
  source 1..30: mol_type = other DNA
tacactttcgggtaccgtaagggctgcttc

SEQ ID NO: 95 - DNA, 30 bp, synthetic construct
  misc_feature 1..30: note = primer
  source 1..30: mol_type = other DNA
taccgtaagggctgcttcggcatcgtcctc

SEQ ID NO: 96 - DNA, 30 bp, synthetic construct
  misc_feature 1..30: note = primer
  source 1..30: mol_type = other DNA
tgcttcggcatcgtcctcgccccaacgctg

SEQ ID NO: 97 - DNA, 30 bp, synthetic construct
  misc_feature 1..30: note = primer
  source 1..30: mol_type = other DNA
gtcctcgccccaacgctggtagtattcata

SEQ ID NO: 98 - DNA, 30 bp, synthetic construct
  misc_feature 1..30: note = primer
  source 1..30: mol_type = other DNA
gccccaacgctggtagtattcatacaggcc

SEQ ID NO: 99 - DNA, 42 bp, synthetic construct
  misc_feature 1..42: note = primer
  source 1..42: mol_type = other DNA
gaaggagatatacatatgaatgaaatgacctacgagcaattg

SEQ ID NO: 100 - DNA, 36 bp, synthetic construct
  misc_feature 1..36: note = primer
  source 1..36: mol_type = other DNA
tcctttcgggctttgttaagaagttaacgcctcctc

SEQ ID NO: 101 - DNA, 30 bp, synthetic construct
  misc_feature 1..30: note = primer
  source 1..30: mol_type = other DNA
caaagcccgaaaggaagctgagttggctgc

SEQ ID NO: 102 - DNA, 36 bp, synthetic construct; identical to SEQ ID NO: 100
  misc_feature 1..36: note = primer
  source 1..36: mol_type = other DNA

SEQ ID NO: 103 - DNA, 30 bp, synthetic construct
  misc_feature 1..30: note = primer
  source 1..30: mol_type = other DNA
attcgtacggatccaggtgtgattacgttt

SEQ ID NO: 104 - DNA, 27 bp, synthetic construct
  misc_feature 1..27: note = primer
  source 1..27: mol_type = other DNA
atccgtacgaatggcgaacaagtacgc

SEQ ID NO: 105 - DNA, 30 bp, synthetic construct
  misc_feature 1..30: note = primer
  source 1..30: mol_type = other DNA
atccgtacgaatgcggaacaagtacgccgc

SEQ ID NO: 106 - DNA, 30 bp, synthetic construct
  misc_feature 1..30: note = primer
  source 1..30: mol_type = other DNA
atccgtacgaattgcgaacaagtacgccgc

SEQ ID NO: 107 - DNA, 30 bp, synthetic construct
  misc_feature 1..30: note = primer
  source 1..30: mol_type = other DNA
atccgtacgaatctggaacaagtacgccgc

SEQ ID NO: 108 - DNA, 30 bp, synthetic construct
  misc_feature 1..30: note = primer
  source 1..30: mol_type = other DNA
atccgtacgaatatggaacaagtacgccgc

SEQ ID NO: 109 - DNA, 30 bp, synthetic construct
  misc_feature 1..30: note = primer
  source 1..30: mol_type = other DNA
atccgtacgaattttgaacaagtacgccgc

SEQ ID NO: 110 - DNA, 30 bp, synthetic construct
  misc_feature 1..30: note = primer
  source 1..30: mol_type = other DNA
atccgtacgaattatgaacaagtacgccgc

SEQ ID NO: 111 - DNA, 30 bp, synthetic construct
  misc_feature 1..30: note = primer
  source 1..30: mol_type = other DNA
atccgtacgaatagcgaacaagtacgccgc

SEQ ID NO: 112 - DNA, 30 bp, synthetic construct
  misc_feature 1..30: note = primer
  source 1..30: mol_type = other DNA
atccgtacgaataccgaacaagtacgccgc

SEQ ID NO: 113 - DNA, 30 bp, synthetic construct
  misc_feature 1..30: note = primer
  source 1..30: mol_type = other DNA
atccgtacgaataacgaacaagtacgccgc

SEQ ID NO: 114 - DNA, 30 bp, synthetic construct
  misc_feature 1..30: note = primer
  source 1..30: mol_type = other DNA
atccgtacgaatcaggaacaagtacgccgc

SEQ ID NO: 115 - DNA, 30 bp, synthetic construct
  misc_feature 1..30: note = primer
  source 1..30: mol_type = other DNA
atccgtacgaatcatgaacaagtacgccgc

SEQ ID NO: 116 - DNA, 30 bp, synthetic construct
  misc_feature 1..30: note = primer
  source 1..30: mol_type = other DNA
atccgtacgaatgatgaacaagtacgccgc

SEQ ID NO: 117 - skipped